European Patent Application EP 4 435 004 A1, published September 25, 2024. Title: Asthma treatment by blocking IL-13 and TSLP. Applicant: Sanofi. The sequence listing filed with the application follows.

SEQUENCE LISTING (21 sequences)

SEQ ID NO: 1 - protein, 671 aa, synthetic construct
  REGION 1..671: note = SAR443765
DVQLVESGGGVVQPGGSLRLSCAASGRTFSSYRMGWFRQAPGKEREFVAALSGDGYSTYTANSVKGRFTISRDNSKNTVYLQMNSLRPEDTALYYCAAKLQYVSGWSYDYPYWGQGTLVTVSSGGGGSGGGGSGGGGSGGGGSGGGGSGGGGSGGGGSEVQLVESGGGVVQPGGSLRLSCAASGFTFNNYAMKWVRQAPGKGLEWVSSITTGGGSTDYADSVKGRFTISRDNSKNTLYLQMNSLRPEDTALYYCANVPFGYYSEHFSGLSFDYRGQGTLVTVSSGGGGSGGGSEVQLVESGGGVVQPGGSLRLSCAASGSGFGVNILYWYRQAAGIERELIASITSGGITNYVDSVKGRFTISRDNSENTMYLQMNSLRAEDTGLYYCASRNIFDGTTEWGQGTLVTVSSGGGGSGGGSEVQLVESGGGVVQPGGSLRLSCAASGFTFRSFGMSWVRQAPGKGPEWVSSISGSGSDTLYADSVKGRFTISRDNSKNTLYLQMNSLRPEDTALYYCTIGGSLSRSSQGTLVTVSSGGGGSGGGSEVQLVESGGGVVQPGGSLRLSCAASGFTFADYDYDIGWFRQAPGKEREGVSCISNRDGSTYYADSVKGRFTISRDNSKNTVYLQMNSLRPEDTALYYCAVEIHCDDYGVENFDFDPWGQGTLVTVSSA

SEQ ID NO: 2 - protein, 123 aa, synthetic construct
  REGION 1..123: note = 4B02
DVQLVESGGGVVQPGGSLRLSCAASGRTFSSYRMGWFRQAPGKEREFVAALSGDGYSTYTANSVKGRFTISRDNSKNTVYLQMNSLRPEDTALYYCAAKLQYVSGWSYDYPYWGQGTLVTVSS

SEQ ID NO: 3 - protein, 126 aa, synthetic construct
  REGION 1..126: note = 4B06
EVQLVESGGGVVQPGGSLRLSCAASGFTFNNYAMKWVRQAPGKGLEWVSSITTGGGSTDYADSVKGRFTISRDNSKNTLYLQMNSLRPEDTALYYCANVPFGYYSEHFSGLSFDYRGQGTLVTVSS

SEQ ID NO: 4 - protein, 117 aa, synthetic construct
  REGION 1..117: note = 501A02
EVQLVESGGGVVQPGGSLRLSCAASGSGFGVNILYWYRQAAGIERELIASITSGGITNYVDSVKGRFTISRDNSENTMYLQMNSLRAEDTGLYYCASRNIFDGTTEWGQGTLVTVSS

SEQ ID NO: 5 - protein, 115 aa, synthetic construct
  REGION 1..115: note = ALB23002
EVQLVESGGGVVQPGGSLRLSCAASGFTFRSFGMSWVRQAPGKGPEWVSSISGSGSDTLYADSVKGRFTISRDNSKNTLYLQMNSLRPEDTALYYCTIGGSLSRSSQGTLVTVSS

SEQ ID NO: 6 - protein, 127 aa, synthetic construct
  REGION 1..127: note = 529F10
EVQLVESGGGVVQPGGSLRLSCAASGFTFADYDYDIGWFRQAPGKEREGVSCISNRDGSTYYADSVKGRFTISRDNSKNTVYLQMNSLRPEDTALYYCAVEIHCDDYGVENFDFDPWGQGTLVTVSS

SEQ ID NO: 7 - protein, 10 aa, synthetic construct
  REGION 1..10: note = CDR1
GRTFSSYRMG

SEQ ID NO: 8 - protein, 10 aa, synthetic construct
  REGION 1..10: note = CDR1
GFTFNNYAMK

SEQ ID NO: 9 - protein, 10 aa, synthetic construct
  REGION 1..10: note = CDR1
GSGFGVNILY

SEQ ID NO: 10 - protein, 10 aa, synthetic construct
  REGION 1..10: note = CDR1
GFTFRSFGMS

SEQ ID NO: 11 - protein, 12 aa, synthetic construct
  REGION 1..12: note = CDR1
GFTFADYDYDIG

SEQ ID NO: 12 - protein, 10 aa, synthetic construct
  REGION 1..10: note = CDR2
ALSGDGYSTY

SEQ ID NO: 13 - protein, 10 aa, synthetic construct
  REGION 1..10: note = CDR2
SITTGGGSTD

SEQ ID NO: 14 - protein, 9 aa, synthetic construct
  REGION 1..9: note = CDR2
SITSGGITN

SEQ ID NO: 15 - protein, 10 aa, synthetic construct
  REGION 1..10: note = CDR2
SISGSGSDTL

SEQ ID NO: 16 - protein, 10 aa, synthetic construct
  REGION 1..10: note = CDR2
CISNRDGSTY

SEQ ID NO: 17 - protein, 14 aa, synthetic construct
  REGION 1..14: note = CDR3
KLQYVSGWSYDYPY

SEQ ID NO: 18 - protein, 17 aa, synthetic construct
  REGION 1..17: note = CDR3
VPFGYYSEHFSGLSFDY

SEQ ID NO: 19 - protein, 9 aa, synthetic construct
  REGION 1..9: note = CDR3
RNIFDGTTE

SEQ ID NO: 20 - protein, 6 aa, synthetic construct
  REGION 1..6: note = CDR3
GGSLSR

SEQ ID NO: 21 - protein, 16 aa, synthetic construct
  REGION 1..16: note = CDR3
EIHCDDYGVENFDFDP